European Patent Specification EP 3 802 868 B1, published March 11, 2026. Title: METHOD FOR DETECTING A TANDEM REPEAT. Applicant: Imperial College of Science, Technology and Medicine. The sequence listing filed with the application follows.

SEQUENCE LISTING (24 sequences)

SEQ ID NO: 1 - DNA, 45 bp, Artificial Sequence
  Artificial sequence
taattaggcaactttcattccggatgtgtgctgagccgaataaat

SEQ ID NO: 2 - DNA, 48 bp, Artificial Sequence
  Artificial sequence
actaaggtgtagttccagcataccgtaagtagatctacctaccgtagt

SEQ ID NO: 3 - DNA, 19 bp, Artificial Sequence
  Artificial sequence
caccacttcagagttgtct

SEQ ID NO: 4 - DNA, 25 bp, Artificial Sequence
  Artificial sequence
gtattttatattcacctacctacca

SEQ ID NO: 5 - DNA, 17 bp, Artificial Sequence
  Artificial sequence
cggaccgcgtgattcat

SEQ ID NO: 6 - DNA, 54 bp, Artificial Sequence
  Artificial sequence
taattaggcaactttcattccggatgtgtgctgagaaaaaggaaagttgtctag

SEQ ID NO: 7 - DNA, 48 bp, Artificial Sequence; identical to SEQ ID NO: 2
  Artificial sequence

SEQ ID NO: 8 - DNA, 19 bp, Artificial Sequence
  Artificial sequence
caccacttcagagttgtct

SEQ ID NO: 9 - DNA, 25 bp, Artificial Sequence
  Artificial sequence
gtattttatattcacctacctacca

SEQ ID NO: 10 - DNA, 26 bp, Artificial Sequence
  Artificial sequence
accatacaccctaactcatactacgg

SEQ ID NO: 11 - DNA, 19 bp, Artificial Sequence
  Artificial sequence
caccacttcagagttgtct

SEQ ID NO: 12 - DNA, 25 bp, Artificial Sequence
  Artificial sequence
gtattttatattcacctacctacca

SEQ ID NO: 13 - DNA, 45 bp, Artificial Sequence; identical to SEQ ID NO: 1
  Artificial sequence

SEQ ID NO: 14 - DNA, 48 bp, Artificial Sequence; identical to SEQ ID NO: 2
  Artificial sequence

SEQ ID NO: 15 - DNA, 17 bp, Artificial Sequence
  Artificial sequence
cggaccgcgtgattcat

SEQ ID NO: 16 - DNA, 19 bp, Artificial Sequence
  Artificial sequence
caccacttcagagttgtct

SEQ ID NO: 17 - DNA, 25 bp, Artificial Sequence
  Artificial sequence
gtattttatattcacctacctacca

SEQ ID NO: 18 - DNA, 54 bp, Artificial Sequence; identical to SEQ ID NO: 6
  Artificial sequence

SEQ ID NO: 19 - DNA, 48 bp, Artificial Sequence; identical to SEQ ID NO: 2
  Artificial sequence

SEQ ID NO: 20 - DNA, 26 bp, Artificial Sequence
  Artificial sequence
accatacaccctaactcatactacgg

SEQ ID NO: 21 - DNA, 8 bp, Artificial Sequence
  Artificial sequence
caacagat

SEQ ID NO: 22 - DNA, 45 bp, Artificial Sequence
  Artificial sequence
cttagtgcgccaggcctacacacgactcggcttactttcaacgga

SEQ ID NO: 23 - DNA, 87 bp, Artificial Sequence
  Artificial sequence
caacagatcttagtgcgccaggcctacacacgactcggcttacttagtgcgccaggcctacacacgactcggcttactttcaacgga

SEQ ID NO: 24 - DNA, 99 bp, Artificial Sequence
  Artificial sequence
caacagatcttagtgcgccaggcctacacacgactcggcttactttcaacagatcttagtgcgccaggcctacacacgactcggcttactttcaacgga